European Patent Application EP 4 537 831 A2, published April 16, 2025. Title: Pharmazeutische Zusammensetzungen mit Anti-RANKL-Antikörpern, Kalzium und Vitamin D, geeignet zur Behandlung und/oder Prophylaxe von Erkrankungen des Knochenstoffwechsels und von therapiebedingten Nebenwirkungen wie Hypokalzämien. Applicant: KARL, Cristoph. Application EP, filed May 19, 2017. The sequence listing filed with the application follows.

SEQUENCE LISTING (9 sequences)

SEQ ID NO: 1 - DNA, 1426 bp, Mus musculus
  source 1..1426: mol_type = unassigned DNA
aagcttgaccaccatggagtttgggctgagctggctttttcttgtggctattttaaaaggtgtccagtgtgaggtgcagctgttggagtctgggggaggcttggtacagcctggggggtccctgagactctcctgtgcagcctctggattcacctttagcagctatgccatgagctgggtccgccaggctccagggaaggggctggagtgggtctcaggtattactgggagtggtggtagtacatactacgcagactccgtgaagggccggttcaccatctccagagacaattccaagaacacgctgtatctgcaaatgaacagcctgagagccgaggacacggccgtatattactgtgcgaaagatccagggactacggtgattatgagttggttcgacccctggggccagggaaccctggtcaccgtctcctcagcctccaccaagggcccatcggtcttccccctggcgccctgctccaggagcacctccgagagcacagcggccctgggctgcctggtcaaggactacttccccgaaccggtgacggtgtcgtggaactcaggcgctctgaccagcggcgtgcacaccttcccagctgtcctacagtcctcaggactctactccctcagcagcgtggtgaccgtgccctccagcaacttcggcacccagacctacacctgcaacgtagatcacaagcccagcaacaccaaggtggacaagacagttgagcgcaaatgttgtgtcgagtgcccaccgtgcccagcaccacctgtggcaggaccgtcagtcttcctcttccccccaaaacccaaggacaccctcatgatctcccggacccctgaggtcacgtgcgtggtggtggacgtgagccacgaagaccccgaggtccagttcaactggtacgtggacggcgtggaggtgcataatgccaagacaaagccacgggaggagcagttcaacagcacgttccgtgtggtcagcgtcctcaccgttgtgcaccaggactggctgaacggcaaggagtacaagtgcaaggtctccaacaaaggcctcccagcccccatcgagaaaaccatctccaaaaccaaagggcagccccgagaaccacaggtgtacaccctgcccccatcccgggaggagatgaccaagaaccaggtcagcctgacctgcctggtcaaaggcttctaccccagcgacatcgccgtggagtgggagagcaatgggcagccggagaacaactacaagaccacacctcccatgctggactccgacggctccttcttcctctacagcaagctcaccgtggacaagagcaggtggcagcaggggaacgtcttctcatgctccgtgatgcatgaggctctgcacaaccactacacgcagaacagcctctccctgtctccgggtaaatgataagtcgac

SEQ ID NO: 2 - protein, 467 aa, Mus musculus
MEFGLSWLFLVAILKGVQCEVQLLESGGGLVQPGGSLRLSCAASGFTFSSYAMSWVRQAPGKGLEWVSGITGSGGSTYYADSVKGRFTISRDNSKNTLYLQMNSLRAEDTAVYYCAKDPGTTVIMSWFDPWGQGTLVTVSSASTKGPSVFPLAPCSRSTSESTAALGCLVKDYFPEPVTVSWNSGALTSGVHTFPAVLQSSGLYSLSSVVTVPSSNFGTQTYTCNVDHKPSNTKVDKTVERKCCVECPPCPAPPVAGPSVFLFPPKPKDTLMISRTPEVTCVVVDVSHEDPEVQFNWYVSGVEVHNAKTKPREEQFNSTFRVVSVLTVVHQDWLNGKEYKCKVSNKGLPAPIEKTISKTKGQPREPQVYTLPPSREEMTKNQVSLTCLVKGFYPSDIAVEWESNGQPENNYKTTPPMLDSDGSFFLYSKLTVDKSRWQQGNVFSCSVMHEALHNHYTQKSLSLSPGK

SEQ ID NO: 3 - DNA, 728 bp, Mus musculus
  source 1..728: mol_type = unassigned DNA
tctagaccaccatggaaaccccagcgcagcttctcttcctcctgctactctggctcccagataccaccggagaaattgtgttgacgcagtctccaggcaccctgtctttgtctccaggggaaagagccaccctctcctgtagggccagtcagagtgttcgcggcaggtacttagcctggtaccagcagaaacctggccaggctcccaggctcctcatctatggtgcatccagcagggccactggcatcccagacaggttcagtggcagtgggtctgggacagacttcactctcaccatcagcagactggagcctgaagattttgcagtgttttactgtcagcagtatggtagttcacctcggacgttcggccaagggaccaaggtggaaatcaaacgaactgtggctgcaccatctgtcttcatcttcccgccatctgatgagcagttgaaatctggaactgcctctgttgtgtgcctgctgaataacttctatcccagagaggccaaagtacagtggaaggtggataacgccctccaatcgggtaactcccaggagagtgtcacagagcaggacagcaaggacagcacctacagcctcagcagcaccctgacgctgagcaaagcagactacgagaaacacaaagtctacgcctgcgaagtcacccatcagggcctgagctcgcccgtcacaaagagcttcaacaggggagagtgttgataagtcgac

SEQ ID NO: 4 - protein, 235 aa, Mus musculus
METPAQLLFLLLLWLPDTTGEIVLTQSPGTLSLSPGERATLSCRASQSVRGRYLAWYQQKPGQAPRLLIYGASSRATGIPDRFSGSGSGTDFTLTISRLEPEDFAVFYCQQYGSSPRTFGQGTKVEIKRTVAAPSVFIFPPSDEQLKSGTASVVCLLNNFQPREAKVQWKVDNALQSGNSQESVTEQDSKDSTYSLSSTLTLSKADYEKHKVYACEVTHQGLSSPVTKSFNRGEC

SEQ ID NO: 5 - protein, 122 aa, Mus musculus
EVQLLESGGGLVQPGGSLRLSCAASGFTFSSYAMSWVRQAPGKGLEWVSGITGSGGSTYYADSVKGRFTISRDNSKNTLYLQMSSLRAEDTAVYYCAKDPGTTVIMSWFDPWGQGTLVTVSS

SEQ ID NO: 6 - protein, 108 aa, Mus musculus
EIVLTQSPGTLSLSPGERATLSCRASQSVRGRYLAWYQQKPGQAPRLLIYGASSRATGIPDRFSGSGSGTDFTLTISRLEPEDFAVFYCQQYGSSPRTFGQGTKVEIK

SEQ ID NO: 7 - protein, 317 aa, Homo sapiens
MRRASRDYTKYLRGSEEMGGGPGAPHEGPLHAPPPPAPHQPPAASRSMFVALLGLGLGQVVCSVALFFYFRAQMDPNRISEDGTHCIYRILRLHENADFQDTTLESQDTKLIPDSCRRIKQAFQGAVQKELQHIVGSQHIRAEKAMVDGSWLDLAKRSKLEAQPFAHLTINATDIPSGSHKVSLSSWYHDRGWAKISNMTFSNGKLIVNQDGFYYLYANICFRHHETSGDLATEYLQLMVYVTKTSIKIPSSHTLMKGGSTKYWSGNSEFHFYSINVGGFFKLRSGEEISIEVSNPSLLDPDQDATYFGAFKVRDID

SEQ ID NO: 8 - protein, 452 aa, Homo sapiens
EVQLLESGGGLVQPGGSLRLSCAASGFTFSSYAMSWVRQAPGKGLEWVSGITGSGGSTYYADSVKGRFTISRDNSKNTLYLQMNSLRAEDTAVYYCAKDPGTTVIMSWFDPWGQGTLVTVSSASTKGPSVFPLAPSSKSTSGGTAALGCLVKDYFPEPVTVSWNSGALTSGVHTFPAVLQSSGLYSLSSVVTVPSSSLGTQTYICNVNHKPSNTKVDKKVEPKSCDKTHTCPPCPAPELLGGPSVFLFPPKPKDTLMISRTPEVTCVVVDVSHEDPEVKFNWYVDGVEVHNAKTKPREEQYNSTYRVVSVLTVLHQDWLNGKEYKCKVSNKALPAPIEKTISKAKGQPREPQVYTLPPSRDELTKNQVSLTCLVKGFYPSDIAVEWESNGQPENNYKTTPPVLDSDGSFFLYSKLTVDKSRWQQGNVFSCSVMHEALHNHYTQKSLSLSPGK

SEQ ID NO: 9 - protein, 215 aa, Homo sapiens
EIVLTQSPGTLSLSPGERATLSCRASQSVRGRYLAWYQQKPGQAPRLLIYGASSRATGIPDRFSGSGSGTDFTLTISRLEPEDFAVFYCQQYGSSPRTFGQGTKVEIKRTVAAPSVFIFPPSDEQLKSGTASVVCLLNNFYPREAKVQWKVDNALQSGNSQESVTEQDSKDSTYSLSSTLTLSKADYEKHKVYACEVTHQGLSSPVTKSFNRGEC